European Patent Application EP 4 592 394 A1, published July 30, 2025. Title: Base Editing of Plant Cell Organelle DNA. Applicant: Institute for Basic Science. The sequence listing filed with the application follows.

SEQUENCE LISTING (45 sequences)

SEQ ID NO: 1 - protein, 138 aa, synthetic construct
  REGION 1..138: note = Synthetic Sequence
GSYALGPYQISAPQLPAYNGQTVGTFYYVNDAGGLESKVFSSGGPTPYPNYANAGHVEGQSALFMRDNGISEGLVFHNNPEGTCGFCVNMTETLLPENAKMTVVPPEGAIPVKRGATGETKVFTGNSNSPKSPTKGGC

SEQ ID NO: 2 - protein, 44 aa, synthetic construct
  REGION 1..44: note = Synthetic Sequence
GSYALGPYQISAPQLPAYNGQTVGTFYYVNDAGGLESKVFSSGG

SEQ ID NO: 3 - protein, 94 aa, synthetic construct
  REGION 1..94: note = Synthetic Sequence
PTPYPNYANAGHVEGQSALFMRDNGISEGLVFHNNPEGTCGFCVNMTETLLPENAKMTVVPPEGAIPVKRGATGETKVFTGNSNSPKSPTKGGC

SEQ ID NO: 4 - protein, 108 aa, synthetic construct
  REGION 1..108: note = Synthetic Sequence
GSYALGPYQISAPQLPAYNGQTVGTFYYVNDAGGLESKVFSSGGPTPYPNYANAGHVEGQSALFMRDNGISEGLVFHNNPEGTCGFCVNMTETLLPENAKMTVVPPEG

SEQ ID NO: 5 - protein, 30 aa, synthetic construct
  REGION 1..30: note = Synthetic Sequence
AIPVKRGATGETKVFTGNSNSPKSPTKGGC

SEQ ID NO: 6 - protein, 123 aa, synthetic construct
  REGION 1..123: note = Synthetic Sequence
GIHGVPAAMAERPFQCRICMRNFSDRSNLSRHIRTHTGEKPFACDICGRKFAISSNLNSHTKIHTGSQKPFQCRICMRNFSRSDNLARHIRTHTGEKPFACDICGRKFATSGNLTRHTKIHLR

SEQ ID NO: 7 - protein, 122 aa, synthetic construct
  REGION 1..122: note = Synthetic Sequence
GIHGVPAAMAERPFQCRICMRNFSRSDNLSVHIRTHTGEKPFACDICGRKFAQKINLQVHTKIHTGEKPFQCRICMRNFSRSDVLSEHIRTHTGEKPFACDICGRKFAQRNHRTTHTKIHLR

SEQ ID NO: 8 - protein, 5 aa, synthetic construct
  REGION 1..5: note = Synthetic Sequence
TGEKQ

SEQ ID NO: 9 - protein, 10 aa, synthetic construct
  REGION 1..10: note = Synthetic Sequence
SGAQGSTLDF

SEQ ID NO: 10 - protein, 16 aa, synthetic construct
  REGION 1..16: note = Synthetic Sequence
SGSETPGTSESATPES

SEQ ID NO: 11 - protein, 33 aa, synthetic construct
  REGION 1..33: note = Synthetic Sequence
GSGGSSGGSSGSETPGTSESATPESSGGSSGGS

SEQ ID NO: 12 - protein, 136 aa, synthetic construct
  REGION 1..136: note = Synthetic Sequence
DIADLRTLGYSQQQQEKIKPKVRSTVAQHHEALVGHGFTHAHIVALSQHPAALGTVAVKYQDMIAALPEATHEAIVGVGKQWSGARALEALLTVAGELRGPPLQLDTGQLLKIAKRGGVTAVEAVHAWRNALTGAP

SEQ ID NO: 13 - protein, 137 aa, synthetic construct
  REGION 1..137: note = Synthetic Sequence
DIADLRTLGYSQQQQEKIKPKVRSTVAQHHEALVGHGFTHAHIVALSQHPAALGTVAVKYQDMIAALPEATHEAIVGVGKRGAGARALEALLTVAGELRGPPLQLDTGQLLKIAKRGGVTAVEAVHAWRNALTGAPL

SEQ ID NO: 14 - protein, 41 aa, synthetic construct
  REGION 1..41: note = Synthetic Sequence
SIVAQLSRPDPALAALTNDHLVALACLGGRPALDAVKKGLG

SEQ ID NO: 15 - protein, 41 aa, synthetic construct; identical to SEQ ID NO: 14
  REGION 1..41: note = Synthetic Sequence

SEQ ID NO: 16 - protein, 54 aa, synthetic construct
  REGION 1..54: note = Synthetic Sequence
MDSQLVLSLKLNPSFTPLSPLFPFTPCSSFSPSLRFSSCYSRRLYSPVTVYAAK

SEQ ID NO: 17 - protein, 36 aa, synthetic construct
  REGION 1..36: note = Synthetic Sequence
MFKQASRLLSRSVAAASSKSVTTRAFSTELPSTLDS

SEQ ID NO: 18 - protein, 135 aa, synthetic construct
  REGION 1..135: note = Synthetic Sequence
DLRTLGYSQQQQEKIKPKVRSTVAQHHEALVGHGFTHAHIVALSQHPAALGTVAVKYQDMIAALPEATHEAIVGVGKQWSGARALEALLTVAGELRGPPLQLDTGQLLKIAKRGGVTAVEAVHAWRNALTGAPLN

SEQ ID NO: 19 - protein, 61 aa, synthetic construct
  REGION 1..61: note = Synthetic Sequence
LTPEQVVAIASNGGGKQALESIVAQLSRPDPALAALTNDHLVALACLGGRPALDAVKKGLG

SEQ ID NO: 20 - protein, 166 aa, synthetic construct
  REGION 1..166: note = Synthetic Sequence
SEVEFSHEYWMRHALTLAKRARDEREVPVGAVLVLNNRVIGEGWNRAIGLHDPTAHAEIMALRQGGLVMQNYRLIDATLYVTFEPCVMCAGAMIHSRIGRVVFGVRNSKRGAAGSLMNVLNYPGMNHRVEITEGILADECAALLCDFYRMPRQVFNAQKKAQSSIN

SEQ ID NO: 21 - protein, 110 aa, synthetic construct
  REGION 1..110: note = Synthetic Sequence
GSGSYALGPYQISAPQLPAYNGQTVGTFYYVNDAGGLESKVFSSGGPTPYPNYANAGHVEGQSALFMRDNGISEGLVFHNNPEGTCGFCVNMTETLLPENAKMTVVPPEG

SEQ ID NO: 22 - protein, 32 aa, synthetic construct
  REGION 1..32: note = Synthetic Sequence
GSAIPVKRGATGETKVFTGNSNSPKSPTKGGC

SEQ ID NO: 23 - protein, 578 aa, synthetic construct
  REGION 1..578: note = Synthetic Sequence
LTPAQVVAIASNGGGKQALETVQRLLPVLCQAHGLTPAQVVAIASNNGGKQALETVQRLLPVLCQDHGLTPAQVVAIASNIGGKQALETVQRLLPVLCQDHGLTPDQVVAIASNIGGKQALETVQRLLPVLCQAHGLTPDQVVAIASNIGGKQALETVQRLLPVLCQDHGLTPDQVVAIASNGGGKQALETVQRLLPVLCQAHGLTPAQVVAIASNGGGKQALETVQRLLPVLCQAHGLTPAQVVAIASNNGGKQALETVQRLLPVLCQDHGLTPAQVVAIASNIGGKQALETVQRLLPVLCQAHGLTPDQVVAIASNIGGKQALETVQRLLPVLCQAHGLTPDQVVAIASNIGGKQALETVQRLLPVLCQAHGLTPAQVVAIASHDGGKQALETVQRLLPVLCQAHGLTPAQVVAIASHDGGKQALETVQRLLPVLCQDHGLTPDQVVAIASNIGGKQALETVQRLLPVLCQDHGLTPAQVVAIASNGGGKQALETVQRLLPVLCQAHGLTPEQVVAIASNGGGKQALETVQRLLPVLCQAHGLTPDQVVAIASNGGGKQALETVQRLLPVLCQAHG

SEQ ID NO: 24 - protein, 578 aa, synthetic construct
  REGION 1..578: note = Synthetic Sequence
LTPDQVVAIASNNGGKQALETVQRLLPVLCQAHGLTPAQVVAIASHDGGKQALETVQRLLPVLCQDHGLTPDQVVAIASNGGGKQALETVQRLLPVLCQAHGLTPEQVVAIASNGGGKQALETVQRLLPVLCQAHGLTPDQVVAIASNGGGKQALETVQRLLPVLCQDHGLTPDQVVAIASNIGGKQALETVQRLLPVLCQDHGLTPAQVVAIASNNGGKQALETVQRLLPVLCQDHGLTPAQVVAIASNNGGKQALETVQRLLPVLCQDHGLTPDQVVAIASNGGGKQALETVQRLLPVLCQAHGLTPDQVVAIASNIGGKQALETVQRLLPVLCQDHGLTPAQVVAIASNGGGKQALETVQRLLPVLCQAHGLTPAQVVAIASHDGGKQALETVQRLLPVLCQDHGLTPAQVVAIASNIGGKQALETVQRLLPVLCQDHGLTPDQVVAIASNNGGKQALETVQRLLPVLCQDHGLTPEQVVAIASHDGGKQALETVQRLLPVLCQAHGLTPEQVVAIASNIGGKQALETVQRLLPVLCQAHGLTPAQVVAIASHDGGKQALETVQRLLPVLCQDHG

SEQ ID NO: 25 - protein, 612 aa, synthetic construct
  REGION 1..612: note = Synthetic Sequence
LTPAQVVAIASNIGGKQALETVQRLLPVLCQDHGLTPDQVVAIASNIGGKQALETVQRLLPVLCQDHGLTPDQVVAIASNNGGKQALETVQRLLPVLCQAHGLTPAQVVAIASNNGGKQALETVQRLLPVLCQAHGLTPDQVVAIASNNGGKQALETVQRLLPVLCQDHGLTPEQVVAIASNNGGKQALETVQRLLPVLCQAHGLTPAQVVAIASHDGGKQALETVQRLLPVLCQDHGLTPDQVVAIASNIGGKQALETVQRLLPVLCQDHGLTPAQVVAIASNGGGKQALETVQRLLPVLCQAHGLTPAQVVAIASNNGGKQALETVQRLLPVLCQDHGLTPAQVVAIASNIGGKQALETVQRLLPVLCQAHGLTPEQVVAIASNGGGKQALETVQRLLPVLCQAHGLTPAQVVAIASNNGGKQALETVQRLLPVLCQDHGLTPAQVVAIASNIGGKQALETVQRLLPVLCQAHGLTPDQVVAIASHDGGKQALETVQRLLPVLCQAHGLTPEQVVAIASNGGGKQALETVQRLLPVLCQAHGLTPAQVVAIASNGGGKQALETVQRLLPVLCQAHGLTPDQVVAIASNNGGKQALETVQRLLPVLCQDHG

SEQ ID NO: 26 - protein, 612 aa, synthetic construct
  REGION 1..612: note = Synthetic Sequence
LTPDQVVAIASNNGGKQALETVQRLLPVLCQAHGLTPDQVVAIASHDGGKQALETVQRLLPVLCQDHGLTPDQVVAIASHDGGKQALETVQRLLPVLCQAHGLTPAQVVAIASNNGGKQALETVQRLLPVLCQDHGLTPAQVVAIASNNGGKQALETVQRLLPVLCQDHGLTPDQVVAIASNGGGKQALETVQRLLPVLCQAHGLTPAQVVAIASNNGGKQALETVQRLLPVLCQDHGLTPAQVVAIASNIGGKQALETVQRLLPVLCQAHGLTPEQVVAIASNGGGKQALETVQRLLPVLCQAHGLTPAQVVAIASNIGGKQALETVQRLLPVLCQDHGLTPDQVVAIASNIGGKQALETVQRLLPVLCQDHGLTPDQVVAIASNNGGKQALETVQRLLPVLCQAHGLTPAQVVAIASHDGGKQALETVQRLLPVLCQDHGLTPDQVVAIASHDGGKQALETVQRLLPVLCQAHGLTPEQVVAIASNNGGKQALETVQRLLPVLCQAHGLTPDQVVAIASNNGGKQALETVQRLLPVLCQDHGLTPAQVVAIASNIGGKQALETVQRLLPVLCQAHGLTPEQVVAIASNNGGKQALETVQRLLPVLCQAHG

SEQ ID NO: 27 - protein, 612 aa, synthetic construct
  REGION 1..612: note = Synthetic Sequence
LTPAQVVAIASHDGGKQALETVQRLLPVLCQAHGLTPAQVVAIASNGGGKQALETVQRLLPVLCQDHGLTPDQVVAIASNNGGKQALETVQRLLPVLCQDHGLTPAQVVAIASNNGGKQALETVQRLLPVLCQDHGLTPEQVVAIASNGGGKQALETVQRLLPVLCQAHGLTPAQVVAIASNGGGKQALETVQRLLPVLCQDHGLTPAQVVAIASHDGGKQALETVQRLLPVLCQDHGLTPDQVVAIASHDGGKQALETVQRLLPVLCQAHGLTPEQVVAIASNNGGKQALETVQRLLPVLCQAHGLTPAQVVAIASNNGGKQALETVQRLLPVLCQAHGLTPDQVVAIASHDGGKQALETVQRLLPVLCQDHGLTPAQVVAIASNNGGKQALETVQRLLPVLCQAHGLTPDQVVAIASNIGGKQALETVQRLLPVLCQAHGLTPDQVVAIASNIGGKQALETVQRLLPVLCQAHGLTPAQVVAIASHDGGKQALETVQRLLPVLCQAHGLTPEQVVAIASNNGGKQALETVQRLLPVLCQAHGLTPDQVVAIASNIGGKQALETVQRLLPVLCQDHGLTPDQVVAIASNIGGKQALETVQRLLPVLCQAHG

SEQ ID NO: 28 - protein, 612 aa, synthetic construct
  REGION 1..612: note = Synthetic Sequence
LTPEQVVAIASNNGGKQALETVQRLLPVLCQAHGLTPDQVVAIASNGGGKQALETVQRLLPVLCQDHGLTPAQVVAIASNNGGKQALETVQRLLPVLCQAHGLTPEQVVAIASNGGGKQALETVQRLLPVLCQAHGLTPAQVVAIASNGGGKQALETVQRLLPVLCQAHGLTPDQVVAIASNNGGKQALETVQRLLPVLCQDHGLTPAQVVAIASNGGGKQALETVQRLLPVLCQDHGLTPAQVVAIASHDGGKQALETVQRLLPVLCQAHGLTPEQVVAIASHDGGKQALETVQRLLPVLCQAHGLTPAQVVAIASNNGGKQALETVQRLLPVLCQAHGLTPDQVVAIASNNGGKQALETVQRLLPVLCQDHGLTPAQVVAIASNIGGKQALETVQRLLPVLCQAHGLTPAQVVAIASNIGGKQALETVQRLLPVLCQDHGLTPDQVVAIASNIGGKQALETVQRLLPVLCQDHGLTPDQVVAIASNNGGKQALETVQRLLPVLCQAHGLTPAQVVAIASNIGGKQALETVQRLLPVLCQAHGLTPAQVVAIASNNGGKQALETVQRLLPVLCQDHGLTPAQVVAIASNNGGKQALETVQRLLPVLCQAHG

SEQ ID NO: 29 - protein, 612 aa, synthetic construct
  REGION 1..612: note = Synthetic Sequence
LTPDQVVAIASNNGGKQALETVQRLLPVLCQAHGLTPDQVVAIASHDGGKQALETVQRLLPVLCQDHGLTPDQVVAIASHDGGKQALETVQRLLPVLCQAHGLTPDQVVAIASNNGGKQALETVQRLLPVLCQDHGLTPAQVVAIASNIGGKQALETVQRLLPVLCQAHGLTPEQVVAIASNNGGKQALETVQRLLPVLCQAHGLTPAQVVAIASNIGGKQALETVQRLLPVLCQDHGLTPAQVVAIASNGGGKQALETVQRLLPVLCQDHGLTPDQVVAIASNIGGKQALETVQRLLPVLCQAHGLTPEQVVAIASNIGGKQALETVQRLLPVLCQAHGLTPAQVVAIASNGGGKQALETVQRLLPVLCQAHGLTPAQVVAIASNNGGKQALETVQRLLPVLCQDHGLTPDQVVAIASNNGGKQALETVQRLLPVLCQAHGLTPDQVVAIASHDGGKQALETVQRLLPVLCQDHGLTPDQVVAIASHDGGKQALETVQRLLPVLCQAHGLTPEQVVAIASNGGGKQALETVQRLLPVLCQAHGLTPDQVVAIASNIGGKQALETVQRLLPVLCQAHGLTPAQVVAIASHDGGKQALETVQRLLPVLCQDHG

SEQ ID NO: 30 - protein, 612 aa, synthetic construct
  REGION 1..612: note = Synthetic Sequence
LTPDQVVAIASNIGGKQALETVQRLLPVLCQDHGLTPAQVVAIASNGGGKQALETVQRLLPVLCQAHGLTPAQVVAIASHDGGKQALETVQRLLPVLCQDHGLTPDQVVAIASNIGGKQALETVQRLLPVLCQAHGLTPDQVVAIASNIGGKQALETVQRLLPVLCQDHGLTPDQVVAIASNGGGKQALETVQRLLPVLCQAHGLTPDQVVAIASNIGGKQALETVQRLLPVLCQAHGLTPDQVVAIASNIGGKQALETVQRLLPVLCQAHGLTPAQVVAIASHDGGKQALETVQRLLPVLCQAHGLTPAQVVAIASNIGGKQALETVQRLLPVLCQDHGLTPDQVVAIASNNGGKQALETVQRLLPVLCQDHGLTPEQVVAIASHDGGKQALETVQRLLPVLCQAHGLTPEQVVAIASNNGGKQALETVQRLLPVLCQAHGLTPDQVVAIASNGGGKQALETVQRLLPVLCQDHGLTPAQVVAIASNNGGKQALETVQRLLPVLCQAHGLTPAQVVAIASHDGGKQALETVQRLLPVLCQDHGLTPDQVVAIASNIGGKQALETVQRLLPVLCQDHGLTPAQVVAIASNGGGKQALETVQRLLPVLCQAHG

SEQ ID NO: 31 - protein, 612 aa, synthetic construct
  REGION 1..612: note = Synthetic Sequence
LTPDQVVAIASNNGGKQALETVQRLLPVLCQAHGLTPAQVVAIASHDGGKQALETVQRLLPVLCQDHGLTPDQVVAIASNGGGKQALETVQRLLPVLCQAHGLTPAQVVAIASHDGGKQALETVQRLLPVLCQDHGLTPEQVVAIASNIGGKQALETVQRLLPVLCQAHGLTPAQVVAIASNIGGKQALETVQRLLPVLCQDHGLTPEQVVAIASNNGGKQALETVQRLLPVLCQAHGLTPDQVVAIASNGGGKQALETVQRLLPVLCQDHGLTPAQVVAIASNNGGKQALETVQRLLPVLCQAHGLTPEQVVAIASNNGGKQALETVQRLLPVLCQAHGLTPAQVVAIASNNGGKQALETVQRLLPVLCQDHGLTPDQVVAIASHDGGKQALETVQRLLPVLCQDHGLTPAQVVAIASNGGGKQALETVQRLLPVLCQAHGLTPDQVVAIASNNGGKQALETVQRLLPVLCQAHGLTPAQVVAIASNGGGKQALETVQRLLPVLCQDHGLTPEQVVAIASNGGGKQALETVQRLLPVLCQAHGLTPAQVVAIASNNGGKQALETVQRLLPVLCQDHGLTPDQVVAIASNNGGKQALETVQRLLPVLCQDHG

SEQ ID NO: 32 - protein, 612 aa, synthetic construct
  REGION 1..612: note = Synthetic Sequence
LTPDQVVAIASNIGGKQALETVQRLLPVLCQDHGLTPDQVVAIASHDGGKQALETVQRLLPVLCQDHGLTPAQVVAIASNIGGKQALETVQRLLPVLCQAHGLTPAQVVAIASNNGGKQALETVQRLLPVLCQAHGLTPDQVVAIASNNGGKQALETVQRLLPVLCQDHGLTPEQVVAIASNNGGKQALETVQRLLPVLCQAHGLTPEQVVAIASNIGGKQALETVQRLLPVLCQAHGLTPAQVVAIASNGGGKQALETVQRLLPVLCQAHGLTPAQVVAIASNNGGKQALETVQRLLPVLCQAHGLTPDQVVAIASNIGGKQALETVQRLLPVLCQAHGLTPAQVVAIASNIGGKQALETVQRLLPVLCQDHGLTPAQVVAIASNIGGKQALETVQRLLPVLCQAHGLTPAQVVAIASNGGGKQALETVQRLLPVLCQAHGLTPAQVVAIASNNGGKQALETVQRLLPVLCQDHGLTPAQVVAIASNIGGKQALETVQRLLPVLCQDHGLTPDQVVAIASNIGGKQALETVQRLLPVLCQAHGLTPAQVVAIASNIGGKQALETVQRLLPVLCQDHGLTPAQVVAIASNIGGKQALETVQRLLPVLCQAHG

SEQ ID NO: 33 - DNA, 138 bp, synthetic construct
  misc_feature 1..138: note = Synthetic Sequence
  source 1..138: mol_type = other DNA
ggctctggttcctacgccctgggtccatatcagattagtgctccccaactccccgcctacaacggtcagacagtggggaccttttactatgtcaacgacgccgggggattggaatccaaggttttctctagcggtggg

SEQ ID NO: 34 - DNA, 282 bp, synthetic construct
  misc_feature 1..282: note = Synthetic Sequence
  source 1..282: mol_type = other DNA
ccaacaccttatcctaactacgctaacgccgggcacgtcgaggggcagtcagctctttttatgagagataacggcattagcgaagggcttgtgttccataataatcctgagggcacctgtggcttctgtgtaaatatgaccgaaacacttctgcctgagaacgctaaaatgactgtcgtaccacccgaaggcgcaatcccagttaaacggggcgcaaccggcgaaaccaaagtattcaccggaaacagcaatagtccaaagtcccccaccaagggaggttgc

SEQ ID NO: 35 - DNA, 324 bp, synthetic construct
  misc_feature 1..324: note = Synthetic Sequence
  source 1..324: mol_type = other DNA
ggtagctacgcacttggtccttaccagattagcgcaccccaactccccgcctataatggtcaaaccgtcgggaccttttactacgtaaacgatgctggtgggctggaatccaaagtattctcctcagggggccctacaccctaccccaactacgccaatgctggtcatgtagaagggcagtcagcactgtttatgcgcgataatggtataagcgaggggttggtcttccataacaacccagagggtacttgtggcttctgtgtgaatatgactgaaacccttctgcccgaaaatgccaagatgactgtcgtcccacctgaaggc

SEQ ID NO: 36 - DNA, 90 bp, synthetic construct
  misc_feature 1..90: note = Synthetic Sequence
  source 1..90: mol_type = other DNA
gccatacctgtgaagcggggagcaacaggggagacaaaggtgttcacaggcaactctaacagtccaaagagccccaccaaaggcgggtgt

SEQ ID NO: 37 - DNA, 408 bp, synthetic construct
  misc_feature 1..408: note = Synthetic Sequence
  source 1..408: mol_type = other DNA
gatatagctgatttgaggaccctcgggtactcacagcagcaacaagaaaaaatcaaaccaaaggtacgtagcacggttgcccaacatcatgaagccctagttggtcacggatttactcatgcccatattgttgcactgagtcaacaccctgctgcattaggcacagtggctgtgaaatatcaagatatgattgctgctcttcctgaggccacacacgaggcaattgtgggtgttggaaaacaatggtctggtgcgcgagcgcttgaagctctcctaaccgtagctggagagttgagaggcccaccgcttcagcttgacacagggcagctgttgaagatagcaaagagggggggtgtaactgctgttgaagcagtccatgcatggagaaatgcattaactggagctcca

SEQ ID NO: 38 - DNA, 411 bp, synthetic construct
  misc_feature 1..411: note = Synthetic Sequence
  source 1..411: mol_type = other DNA
gatattgctgatcttcgaacattgggttattctcagcagcaacaagagaaaatcaaaccgaaagtccgttcaaccgtagctcaacatcatgaagcccttgttggtcatggatttactcatgctcacattgttgctctaagtcagcaccctgccgcgctaggcacagttgccgtcaagtatcaagatatgatagctgctttacctgaagcaacccacgaggcaatagtgggggttgggaagaggggtgcaggcgccagggcactggaggcactcttaacagtagctggagaacttcggggaccaccattgcagcttgatactggacaactcttgaagatcgcaaaaagagggggtgtgactgctgtggaagctgttcatgcatggagaaatgctttgacgggagcacccctg

SEQ ID NO: 39 - DNA, 123 bp, synthetic construct
  misc_feature 1..123: note = Synthetic Sequence
  source 1..123: mol_type = other DNA
agcatagttgctcagctaagtagacctgatccagcacttgctgcattgacgaacgatcatctcgtagcgctggcttgtttgggcggcaggccagccttggacgccgtgaagaaaggattaggt

SEQ ID NO: 40 - DNA, 123 bp, synthetic construct
  misc_feature 1..123: note = Synthetic Sequence
  source 1..123: mol_type = other DNA
tcgatagtagcacaattaagcaggcctgaccctgcacttgctgctcttacaaatgatcatcttgttgctctggcctgtttgggtgggcgtcccgcgttggatgctgttaagaaaggacttggt

SEQ ID NO: 41 - DNA, 1660 bp, synthetic construct
  misc_feature 1..1660: note = Synthetic Sequence
  source 1..1660: mol_type = other DNA
ctcaacttttgattcgctatttgcagtgcacctgtggcgttcatcacatcttttgtgacactgtttgcactggtcattgctattacaaaggaccttcctgatgttgaaggagatcgaaagtaagtaactgcacgcataaccattttctttccgctctttggctcaatccatttgacagtcaaagacaatgtttaaccagctccgtttgatatattgtctttatgtgtttgttcaagcatgtttagttaatcatgcctttgattgatcttgaataggttccaaatatcaaccctggcaacaaaacttggagtgagaaacattgcattcctcggttctggacttctgctagtaaattatgtttcagccatatcactagctttctacatgcctcaggtgaattcatctatttccgtcttaactatttcggttaattaaagcacgaacaccattactgcatgtagaagcttgataaactatcgccaccaatttatttttgttgcgatattgttactttcctcagtatgcagctttgaaaagaccaaccctcttatcctttaacaatgaacaggtttttagaggtagcttgatgattcctgcacatgtgatcttggcttcaggcttaattttccaggtaaagcattatgagatactcttatatctcttacatacttttgagataatgcacaagaacttcataactatatgctttagtttctgcatttgacactgccaaattcattaatctctaatatctttgttgttgatctttggtagacatgggtactagaaaaagcaaactacaccaaggtaaaatacttttgtacaaacataaactcgttatcacggaacatcaatggagtgtatatctaacggagtgtagaaacatttgattattgcaggaagctatctcaggatattatcggtttatatggaatctcttctacgcagagtatctgttattccccttcctctagctttcaatttcatggtgaggatatgcagttttctttgtatatcattcttcttcttctttgtagcttggagtcaaaatcggttccttcatgtacatacatcaaggatatgtccttctgaatttttatatcttgcaataaaaatgcttgtaccaattgaaacaccagctttttgagttctatgatcactgacttggttctaaccaaaaaaaaaaaaatgtttaatttacatatctaaaagtaggtttagggaaacctaaacagtaaaatatttgtatattattcgaatttcactcatcataaaaacttaaattgcaccataaaattttgttttactattaatgatgtaatttgtgtaacttaagataaaaataatattccgtaagttaaccggctaaaaccacgtataaaccagggaacctgttaaaccggttctttactggataaagaaatgaaagcccatgtagacagctccattagagcccaaaccctaaatttctcatctatataaaaggagtgacattagggtttttgttcgtcctcttaaagcttctcgttttctctgccgtctctctcattcgcgcgacgcaaacgatcttcaggtgatcttctttctccaaatcctctctcataactctgatttcgtacttgtgtatttgagctcacgctctgtttctctcaccacagcc

SEQ ID NO: 42 - DNA, 1660 bp, synthetic construct; identical to SEQ ID NO: 41
  misc_feature 1..1660: note = Synthetic Sequence
  source 1..1660: mol_type = other DNA

SEQ ID NO: 43 - DNA, 917 bp, synthetic construct
  misc_feature 1..917: note = Synthetic Sequence
  source 1..917: mol_type = other DNA
ctagcaacgattgtacaattgcttctttaaaaaaggaagaaagaaagaaagaaaagaatcaacatcagcgttaacaaacggccccgttacggcccaaacggtcatatagagtaacggcgttaagcgttgaaagactcctatcgaaatacgtaaccgcaaacgtgtcatagtcagatcccctcttccttcaccgcctcaaacacaaaaataatcttctacagcctatatatacaacccccccttctatctctcctttctcacaattcatcatctttctttctctacccccaattttaagaaatcctctcttctcctcttcattttcaaggtaaatctctctctctctctctctctctgttattccttgttttaattaggtatgtattattgctagtttgttaatctgcttatcttatgtatgccttatgtgaatatctttatcttgttcatctcatccgtttagaagctataaatttgttgatttgactgtgtatctacacgtggttatgtttatatctaatcagatatgaatttcttcatattgttgcgtttgtgtgtaccaatccgaaatcgttgatttttttcatttaatcgtgtagctaattgtacgtatacatatggatctacgtatcaattgttcatctgtttgtgtttgtatgtatacagatctgaaaacatcacttctctcatctgattgtgttgttacatacatagatatagatctgttatatcattttttttattaattgtgtatatatatatgtgcatagatctggattacatgattgtgattatttacatgattttgttatttacgtatgtatatatgtagatctggactttttggagttgttgacttgattgtatttgtgtgtgtatatgtgtgttctgatcttgatatgttatgtatgtgcagc

SEQ ID NO: 44 - DNA, 469 bp, synthetic construct
  misc_feature 1..469: note = Synthetic Sequence
  source 1..469: mol_type = other DNA
caggcctcccagctttcgtccgtatcatcggtttcgacaacgttcgtcaagttcaatgcatcagtttcattgcccacacaccagaatcctactaagtttgagtattatggcattggaaaagctgttttcttctatcatttgttctgcttgtaatttactgtgttctttcagtttttgttttcggacatcaaaatgcaaatggatggataagagttaataaatgatatggtccttttgttcattctcaaattattattatctgttgtttttactttaatgggttgaatttaagtaagaaaggaactaacagtgtgatattaaggtgcaatgttagacatataaaacagtctttcacctctctttggttatgtcttgaattggtttgtttcttcacttatctgtgtaatcaagtttactatgagtctatgatcaagtaattatgcaatcaagttaagtacagtataggctt

SEQ ID NO: 45 - protein, 24 aa, synthetic construct
  REGION 1..24: note = Synthetic Sequence
SGTPHEVGVYTLSGTPHEVGVYTL